European Patent Application EP 4 205 762 A1, published July 5, 2023. Title: Improved DNA vaccine for SARS-CoV-2. Applicant: OSAKA UNIVERSITY TAKARA BIO INC. AnGes, Inc. The sequence listing filed with the application follows.

SEQUENCE LISTING (18 sequences)

SEQ ID NO: 1 - protein, 1273 aa, SARS-CoV-2
MFVFLVLLPLVSSQCVNLTTRTQLPPAYTNSFTRGVYYPDKVFRSSVLHSTQDLFLPFFSNVTWFHAIHVSGTNGTKRFDNPVLPFNDGVYFASTEKSNIIRGWIFGTTLDSKTQSLLIVNNATNVVIKVCEFQFCNDPFLGVYYHKNNKSWMESEFRVYSSANNCTFEYVSQPFLMDLEGKQGNFKNLREFVFKNIDGYFKIYSKHTPINLVRDLPQGFSALEPLVDLPIGINITRFQTLLALHRSYLTPGDSSSGWTAGAAAYYVGYLQPRTFLLKYNENGTITDAVDCALDPLSETKCTLKSFTVEKGIYQTSNFRVQPTESIVRFPNITNLCPFGEVFNATRFASVYAWNRKRISNCVADYSVLYNSASFSTFKCYGVSPTKLNDLCFTNVYADSFVIRGDEVRQIAPGQTGKIADYNYKLPDDFTGCVIAWNSNNLDSKVGGNYNYLYRLFRKSNLKPFERDISTEIYQAGSTPCNGVEGFNCYFPLQSYGFQPTNGVGYQPYRVVVLSFELLHAPATVCGPKKSTNLVKNKCVNFNFNGLTGTGVLTESNKKFLPFQQFGRDIADTTDAVRDPQTLEILDITPCSFGGVSVITPGTNTSNQVAVLYQDVNCTEVPVAIHADQLTPTWRVYSTGSNVFQTRAGCLIGAEHVNNSYECDIPIGAGICASYQTQTNSPRRARSVASQSIIAYTMSLGAENSVAYSNNSIAIPTNFTISVTTEILPVSMTKTSVDCTMYICGDSTECSNLLLQYGSFCTQLNRALTGIAVEQDKNTQEVFAQVKQIYKTPPIKDFGGFNFSQILPDPSKPSKRSFIEDLLFNKVTLADAGFIKQYGDCLGDIAARDLICAQKFNGLTVLPPLLTDEMIAQYTSALLAGTITSGWTFGAGAALQIPFAMQMAYRFNGIGVTQNVLYENQKLIANQFNSAIGKIQDSLSSTASALGKLQDVVNQNAQALNTLVKQLSSNFGAISSVLNDILSRLDKVEAEVQIDRLITGRLQSLQTYVTQQLIRAAEIRASANLAATKMSECVLGQSKRVDFCGKGYHLMSFPQSAPHGVVFLHVTYVPAQEKNFTTAPAICHDGKAHFPREGVFVSNGTHWFVTQRNFYEPQIITTDNTFVSGNCDVVIGIVNNTVYDPLQPELDSFKEELDKYFKNHTSPDVDLGDISGINASVVNIQKEIDRLNEVAKNLNESLIDLQELGKYEQYIKWPWYIWLGFIAGLIAIVMVTIMLCCMTSCCSCLKGCCSCGSCCKFDEDDSEPVLKGVKLHYT

SEQ ID NO: 2 - DNA, 3822 bp, SARS-CoV-2
atgtttgtttttcttgttttattgccactagtctctagtcagtgtgttaatcttacaaccagaactcaattaccccctgcatacactaattctttcacacgtggtgtttattaccctgacaaagttttcagatcctcagttttacattcaactcaggacttgttcttacctttcttttccaatgttacttggttccatgctatacatgtctctgggaccaatggtactaagaggtttgataaccctgtcctaccatttaatgatggtgtttattttgcttccactgagaagtctaacataataagaggctggatttttggtactactttagattcgaagacccagtccctacttattgttaataacgctactaatgttgttattaaagtctgtgaatttcaattttgtaatgatccatttttgggtgtttattaccacaaaaacaacaaaagttggatggaaagtgagttcagagtttattctagtgcgaataattgcacttttgaatatgtctctcagccttttcttatggaccttgaaggaaaacagggtaatttcaaaaatcttagggaatttgtgtttaagaatattgatggttattttaaaatatattctaagcacacgcctattaatttagtgcgtgatctccctcagggtttttcggctttagaaccattggtagatttgccaataggtattaacatcactaggtttcaaactttacttgctttacatagaagttatttgactcctggtgattcttcttcaggttggacagctggtgctgcagcttattatgtgggttatcttcaacctaggacttttctattaaaatataatgaaaatggaaccattacagatgctgtagactgtgcacttgaccctctctcagaaacaaagtgtacgttgaaatccttcactgtagaaaaaggaatctatcaaacttctaactttagagtccaaccaacagaatctattgttagatttcctaatattacaaacttgtgcccttttggtgaagtttttaacgccaccagatttgcatctgtttatgcttggaacaggaagagaatcagcaactgtgttgctgattattctgtcctatataattccgcatcattttccacttttaagtgttatggagtgtctcctactaaattaaatgatctctgctttactaatgtctatgcagattcatttgtaattagaggtgatgaagtcagacaaatcgctccagggcaaactggaaagattgctgattataattataaattaccagatgattttacaggctgcgttatagcttggaattctaacaatcttgattctaaggttggtggtaattataattacctgtatagattgtttaggaagtctaatctcaaaccttttgagagagatatttcaactgaaatctatcaggccggtagcacaccttgtaatggtgttgaaggttttaattgttactttcctttacaatcatatggtttccaacccactaatggtgttggttaccaaccatacagagtagtagtactttcttttgaacttctacatgcaccagcaactgtttgtggacctaaaaagtctactaatttggttaaaaacaaatgtgtcaatttcaacttcaatggtttaacaggcacaggtgttcttactgagtctaacaaaaagtttctgcctttccaacaatttggcagagacattgctgacactactgatgctgtccgtgatccacagacacttgagattcttgacattacaccatgttcttttggtggtgtcagtgttataacaccaggaacaaatacttctaaccaggttgctgttctttatcaggatgttaactgcacagaagtccctgttgctattcatgcagatcaacttactcctacttggcgtgtttattctacaggttctaatgtttttcaaacacgtgcaggctgtttaataggggctgaacatgtcaacaactcatatgagtgtgacatacccattggtgcaggtatatgcgctagttatcagactcagactaattctcctcggcgggcacgtagtgtagctagtcaatccatcattgcctacactatgtcacttggtgcagaaaattcagttgcttactctaataactctattgccatacccacaaattttactattagtgttaccacagaaattctaccagtgtctatgaccaagacatcagtagattgtacaatgtacatttgtggtgattcaactgaatgcagcaatcttttgttgcaatatggcagtttttgtacacaattaaaccgtgctttaactggaatagctgttgaacaagacaaaaacacccaagaagtttttgcacaagtcaaacaaatttacaaaacaccaccaattaaagattttggtggttttaatttttcacaaatattaccagatccatcaaaaccaagcaagaggtcatttattgaagatctacttttcaacaaagtgacacttgcagatgctggcttcatcaaacaatatggtgattgccttggtgatattgctgctagagacctcatttgtgcacaaaagtttaacggccttactgttttgccacctttgctcacagatgaaatgattgctcaatacacttctgcactgttagcgggtacaatcacttctggttggacctttggtgcaggtgctgcattacaaataccatttgctatgcaaatggcttataggtttaatggtattggagttacacagaatgttctctatgagaaccaaaaattgattgccaaccaatttaatagtgctattggcaaaattcaagactcactttcttccacagcaagtgcacttggaaaacttcaagatgtggtcaaccaaaatgcacaagctttaaacacgcttgttaaacaacttagctccaattttggtgcaatttcaagtgttttaaatgatatcctttcacgtcttgacaaagttgaggctgaagtgcaaattgataggttgatcacaggcagacttcaaagtttgcagacatatgtgactcaacaattaattagagctgcagaaatcagagcttctgctaatcttgctgctactaaaatgtcagagtgtgtacttggacaatcaaaaagagttgatttttgtggaaagggctatcatcttatgtccttccctcagtcagcacctcatggtgtagtcttcttgcatgtgacttatgtccctgcacaagaaaagaacttcacaactgctcctgccatttgtcatgatggaaaagcacactttcctcgtgaaggtgtctttgtttcaaatggcacacactggtttgtaacacaaaggaatttttatgaaccacaaatcattactacagacaacacatttgtgtctggtaactgtgatgttgtaataggaattgtcaacaacacagtttatgatcctttgcaacctgaattagactcattcaaggaggagttagataaatattttaagaatcatacatcaccagatgttgatttaggtgacatctctggcattaatgcttcagttgtaaacattcaaaaagaaattgaccgcctcaatgaggttgccaagaatttaaatgaatctctcatcgatctccaagaacttggaaagtatgagcagtatataaaatggccatggtacatttggctaggttttatagctggcttgattgccatagtaatggtgacaattatgctttgctgtatgaccagttgctgtagttgtctcaagggctgttgttcttgtggatcctgctgcaaatttgatgaagacgactctgagccagtgctcaaaggagtcaaattacattacacataa

SEQ ID NO: 3 - DNA, 3822 bp, Artificial
  Codon-modified DNA sequence coding SARS-CoV-2 spike protein
atgttcgtgttcctggtgctgctgcccctggtgagcagccagtgcgtgaacctgaccaccagaacccagctgccccccgcctacaccaacagcttcaccagaggcgtgtactaccccgacaaggtgttcagaagcagcgtgctgcacagcacccaggacctgttcctgcccttcttcagcaacgtgacctggttccacgccatccacgtgagcggcaccaacggcaccaagagattcgacaaccccgtgctgcccttcaacgacggcgtgtacttcgccagcaccgagaagagcaacatcatcagaggctggatcttcggcaccaccctggacagcaagacccagagcctgctgatcgtgaacaacgccaccaacgtggtgatcaaggtgtgcgagttccagttctgcaacgaccccttcctgggcgtgtactaccacaagaacaacaagagctggatggagagcgagttcagagtgtacagcagcgccaacaactgcaccttcgagtacgtgagccagcccttcctgatggacctggagggcaagcagggcaacttcaagaacctgagagagttcgtgttcaagaacatcgacggctacttcaagatctacagcaagcacacccccatcaacctggtgagagacctgcctcagggctttagcgccctggagccactggtggacctgccaatcggcatcaacatcaccagattccagaccctgctggccctgcacagaagctacctgacaccaggcgattctagctctggatggacagccggcgccgctgcctattacgtgggctacctgcagcctagaaccttcctgctgaagtacaacgagaacggcaccatcaccgatgccgtggactgcgccctggatcccctgagcgagaccaagtgtaccctgaagagcttcaccgtggagaagggcatctaccagaccagcaacttcagagtgcagcccaccgagagcatcgtgagattccccaacatcaccaacctgtgccccttcggcgaggtgttcaacgccaccagattcgccagcgtgtacgcctggaacagaaagagaatcagcaactgcgtggccgactacagcgtgctgtacaacagcgccagcttcagcaccttcaagtgctacggcgtgagccccaccaagctgaacgacctgtgcttcaccaacgtgtacgccgacagcttcgtgatcagaggcgacgaggtgagacagattgcccctggccagaccggcaagatcgccgactacaactacaagctgcccgacgacttcaccggctgcgtgatcgcctggaacagcaacaacctggacagcaaggtgggcggcaactacaactacctgtacagactgttcagaaagagcaacctgaagcccttcgagagagacatcagcaccgagatctaccaggccggctctaccccatgcaatggcgtggagggcttcaattgctacttccccctgcagagctacggcttccagcccaccaacggcgtgggctaccagccctacagagtggtggtgctgagctttgaactgctgcacgcccctgccaccgtgtgcggcccaaagaagagcaccaatctggtgaagaacaagtgcgtgaacttcaacttcaacggcctgaccggcaccggcgtgctgaccgagagcaacaagaagttcctgcccttccagcagttcggcagagacatcgccgacaccaccgatgccgtgagagatccccagaccctggagatcctggacatcaccccctgtagctttggcggcgtgagcgtgattacccccggcaccaataccagcaaccaggtggccgtgctgtaccaggacgtgaactgcaccgaggtgccagtggccatccatgccgaccagctgaccccaacctggagagtgtacagcaccggcagcaacgtgttccagacaagagccggctgtctgattggcgccgagcacgtgaataacagctacgagtgcgatatcccaatcggcgccggcatctgtgccagctatcagacccagaccaatagccccagaagagccagaagcgtggccagccagagcatcatcgcctacaccatgagcctgggcgccgagaacagcgtggcctacagcaacaacagcatcgccatccccaccaacttcaccatcagcgtgaccaccgagatcctgcccgtgagcatgaccaagaccagcgtggactgcaccatgtacatctgcggcgacagcaccgagtgcagcaacctgctgctgcagtacggcagcttctgcacccagctgaacagagccctgaccggcatcgccgtggagcaggacaagaacacccaggaggtgttcgcccaggtgaagcagatctacaagaccccccccatcaaggacttcggcggcttcaacttcagccagatcctgcccgaccccagcaagcccagcaagagaagcttcatcgaggacctgctgttcaacaaggtgaccctggccgacgccggcttcatcaagcagtacggcgactgcctgggcgacatcgccgccagagacctgatctgcgcccagaagtttaatggactgacagtgctgccacccctgctgaccgatgagatgatcgcccagtacaccagcgctctgctggccggcacaatcaccagcggctggacatttggagccggagccgctctgcagatcccatttgccatgcagatggcctacagattcaacggcatcggcgtgacccagaacgtgctgtacgagaaccagaagctgatcgccaaccagttcaacagcgccatcggcaagatccaggacagcctgtctagcacagcctctgccctgggcaagctgcaggatgtggtgaaccagaacgcccaggccctgaacaccctggtgaagcagctgagcagcaacttcggcgccatcagcagcgtgctgaacgacatcctgagcagactggacaaggtggaggccgaggtgcagatcgacagactgatcaccggcagactgcagagcctgcagacctacgtgacccagcagctgatcagagccgccgaaatcagagccagcgccaatctggccgccaccaagatgagcgagtgcgtgctgggccagagcaagagagtggacttctgcggcaagggctaccacctgatgagctttccccagagcgcccctcacggcgtggtgtttctgcacgtgacctacgtgcctgcccaggagaagaacttcaccaccgcccctgccatctgccacgatggcaaggcccacttccctagagagggcgtgttcgtgagcaacggcacccactggttcgtgacccagagaaacttctacgagccccagatcatcaccaccgacaacaccttcgtgagcggcaactgcgacgtggtgatcggcatcgtgaacaacaccgtgtacgaccccctgcagcccgagctggacagcttcaaggaggagctggacaagtacttcaagaaccacaccagccccgatgtggacctgggcgatatcagcggcatcaatgccagcgtggtgaacatccagaaggagatcgaccggctcaatgaggtggccaagaacctgaacgagagcctgatcgacctgcaggaactgggcaaatatgagcagtacatcaagtggccctggtacatctggctgggcttcatcgccggcctgatcgccatcgtgatggtgaccatcatgctgtgctgcatgaccagctgctgcagctgcctgaagggctgctgcagctgcgggtcttgttgcaagttcgacgaggacgacagcgagcccgtgctgaagggcgtgaagctgcactacacctaa

SEQ ID NO: 4 - DNA, 6734 bp, Artificial
  Plasmid CO
gctgcttcgcgatgtacgggccagatatacgcgttgacattgattattgactagttattaatagtaatcaattacggggtcattagttcatagcccatatatggagttccgcgttacataacttacggtaaatggcccgcctggctgaccgcccaacgacccccgcccattgacgtcaataatgacgtatgttcccatagtaacgccaatagggactttccattgacgtcaatgggtggagtatttacggtaaactgcccacttggcagtacatcaagtgtatcatatgccaagtacgccccctattgacgtcaatgacggtaaatggcccgcctggcattatgcccagtacatgaccttatgggactttcctacttggcagtacatctacgtattagtcatcgctattaccatggtgatgcggttttggcagtacatcaatgggcgtggatagcggtttgactcacggggatttccaagtctccaccccattgacgtcaatgggagtttgttttggcaccaaaatcaacgggactttccaaaatgtcgtaacaactccgccccattgacgcaaatgggcggtaggcgtgtacggtgggaggtctatataagcagagctctctggctaactagagaacccactgcttactggcttatcgaaattaatacgactcactatagggagacccaagctggctagccaccatgttcgtgttcctggtgctgctgcccctggtgagcagccagtgcgtgaacctgaccaccagaacccagctgccccccgcctacaccaacagcttcaccagaggcgtgtactaccccgacaaggtgttcagaagcagcgtgctgcacagcacccaggacctgttcctgcccttcttcagcaacgtgacctggttccacgccatccacgtgagcggcaccaacggcaccaagagattcgacaaccccgtgctgcccttcaacgacggcgtgtacttcgccagcaccgagaagagcaacatcatcagaggctggatcttcggcaccaccctggacagcaagacccagagcctgctgatcgtgaacaacgccaccaacgtggtgatcaaggtgtgcgagttccagttctgcaacgaccccttcctgggcgtgtactaccacaagaacaacaagagctggatggagagcgagttcagagtgtacagcagcgccaacaactgcaccttcgagtacgtgagccagcccttcctgatggacctggagggcaagcagggcaacttcaagaacctgagagagttcgtgttcaagaacatcgacggctacttcaagatctacagcaagcacacccccatcaacctggtgagagacctgcctcagggctttagcgccctggagccactggtggacctgccaatcggcatcaacatcaccagattccagaccctgctggccctgcacagaagctacctgacaccaggcgattctagctctggatggacagccggcgccgctgcctattacgtgggctacctgcagcctagaaccttcctgctgaagtacaacgagaacggcaccatcaccgatgccgtggactgcgccctggatcccctgagcgagaccaagtgtaccctgaagagcttcaccgtggagaagggcatctaccagaccagcaacttcagagtgcagcccaccgagagcatcgtgagattccccaacatcaccaacctgtgccccttcggcgaggtgttcaacgccaccagattcgccagcgtgtacgcctggaacagaaagagaatcagcaactgcgtggccgactacagcgtgctgtacaacagcgccagcttcagcaccttcaagtgctacggcgtgagccccaccaagctgaacgacctgtgcttcaccaacgtgtacgccgacagcttcgtgatcagaggcgacgaggtgagacagattgcccctggccagaccggcaagatcgccgactacaactacaagctgcccgacgacttcaccggctgcgtgatcgcctggaacagcaacaacctggacagcaaggtgggcggcaactacaactacctgtacagactgttcagaaagagcaacctgaagcccttcgagagagacatcagcaccgagatctaccaggccggctctaccccatgcaatggcgtggagggcttcaattgctacttccccctgcagagctacggcttccagcccaccaacggcgtgggctaccagccctacagagtggtggtgctgagctttgaactgctgcacgcccctgccaccgtgtgcggcccaaagaagagcaccaatctggtgaagaacaagtgcgtgaacttcaacttcaacggcctgaccggcaccggcgtgctgaccgagagcaacaagaagttcctgcccttccagcagttcggcagagacatcgccgacaccaccgatgccgtgagagatccccagaccctggagatcctggacatcaccccctgtagctttggcggcgtgagcgtgattacccccggcaccaataccagcaaccaggtggccgtgctgtaccaggacgtgaactgcaccgaggtgccagtggccatccatgccgaccagctgaccccaacctggagagtgtacagcaccggcagcaacgtgttccagacaagagccggctgtctgattggcgccgagcacgtgaataacagctacgagtgcgatatcccaatcggcgccggcatctgtgccagctatcagacccagaccaatagccccagaagagccagaagcgtggccagccagagcatcatcgcctacaccatgagcctgggcgccgagaacagcgtggcctacagcaacaacagcatcgccatccccaccaacttcaccatcagcgtgaccaccgagatcctgcccgtgagcatgaccaagaccagcgtggactgcaccatgtacatctgcggcgacagcaccgagtgcagcaacctgctgctgcagtacggcagcttctgcacccagctgaacagagccctgaccggcatcgccgtggagcaggacaagaacacccaggaggtgttcgcccaggtgaagcagatctacaagaccccccccatcaaggacttcggcggcttcaacttcagccagatcctgcccgaccccagcaagcccagcaagagaagcttcatcgaggacctgctgttcaacaaggtgaccctggccgacgccggcttcatcaagcagtacggcgactgcctgggcgacatcgccgccagagacctgatctgcgcccagaagtttaatggactgacagtgctgccacccctgctgaccgatgagatgatcgcccagtacaccagcgctctgctggccggcacaatcaccagcggctggacatttggagccggagccgctctgcagatcccatttgccatgcagatggcctacagattcaacggcatcggcgtgacccagaacgtgctgtacgagaaccagaagctgatcgccaaccagttcaacagcgccatcggcaagatccaggacagcctgtctagcacagcctctgccctgggcaagctgcaggatgtggtgaaccagaacgcccaggccctgaacaccctggtgaagcagctgagcagcaacttcggcgccatcagcagcgtgctgaacgacatcctgagcagactggacaaggtggaggccgaggtgcagatcgacagactgatcaccggcagactgcagagcctgcagacctacgtgacccagcagctgatcagagccgccgaaatcagagccagcgccaatctggccgccaccaagatgagcgagtgcgtgctgggccagagcaagagagtggacttctgcggcaagggctaccacctgatgagctttccccagagcgcccctcacggcgtggtgtttctgcacgtgacctacgtgcctgcccaggagaagaacttcaccaccgcccctgccatctgccacgatggcaaggcccacttccctagagagggcgtgttcgtgagcaacggcacccactggttcgtgacccagagaaacttctacgagccccagatcatcaccaccgacaacaccttcgtgagcggcaactgcgacgtggtgatcggcatcgtgaacaacaccgtgtacgaccccctgcagcccgagctggacagcttcaaggaggagctggacaagtacttcaagaaccacaccagccccgatgtggacctgggcgatatcagcggcatcaatgccagcgtggtgaacatccagaaggagatcgaccggctcaatgaggtggccaagaacctgaacgagagcctgatcgacctgcaggaactgggcaaatatgagcagtacatcaagtggccctggtacatctggctgggcttcatcgccggcctgatcgccatcgtgatggtgaccatcatgctgtgctgcatgaccagctgctgcagctgcctgaagggctgctgcagctgcgggtcttgttgcaagttcgacgaggacgacagcgagcccgtgctgaagggcgtgaagctgcactacacctaatctagagggcccgtttaaacccgctgatcagcctcgactgtgccttctagttgccagccatctgttgtttgcccctcccccgtgccttccttgaccctggaaggtgccactcccactgtcctttcctaataaaatgaggaaattgcatcgcattgtctgagtaggtgtcattctattctggggggtggggtggggcaggacagcaagggggaggattgggaagacaatagcaggcatgctggggatgcggtgggctctatggcttctactgggcggttttatggacagcaagcgaaccggaattgccagctggggcgccctctggtaaggttgggaagccctgcaaagtaaactggatggctttcttgccgccaaggatctgatggcgcaggggatcaagctctgatcaagagacaggatgaggatcgtttcgcatgattgaacaagatggattgcacgcaggttctccggccgcttgggtggagaggctattcggctatgactgggcacaacagacaatcggctgctctgatgccgccgtgttccggctgtcagcgcaggggcgcccggttctttttgtcaagaccgacctgtccggtgccctgaatgaactgcaagacgaggcagcgcggctatcgtggctggccacgacgggcgttccttgcgcagctgtgctcgacgttgtcactgaagcgggaagggactggctgctattgggcgaagtgccggggcaggatctcctgtcatctcaccttgctcctgccgagaaagtatccatcatggctgatgcaatgcggcggctgcatacgcttgatccggctacctgcccattcgaccaccaagcgaaacatcgcatcgagcgagcacgtactcggatggaagccggtcttgtcgatcaggatgatctggacgaagagcatcaggggctcgcgccagccgaactgttcgccaggctcaaggcgagcatgcccgacggcgaggatctcgtcgtgacccatggcgatgcctgcttgccgaatatcatggtggaaaatggccgcttttctggattcatcgactgtggccggctgggtgtggcggaccgctatcaggacatagcgttggctacccgtgatattgctgaagagcttggcggcgaatgggctgaccgcttcctcgtgctttacggtatcgccgctcccgattcgcagcgcatcgccttctatcgccttcttgacgagttcttctgaattattaacgcttacaatttcctgatgcggtattttctccttacgcatctgtgcggtatttcacaccgcatcaggtggcacttttcggggaaatgtgcgcggaacccctatttgtttatttttctaaatacattcaaatatgtatccgctcatgagacaataaccctgataaatgcttcaataatagcacgtgctaaaacttcatttttaatttaaaaggatctaggtgaagatcctttttgataatctcatgaccaaaatcccttaacgtgagttttcgttccactgagcgtcagaccccgtagaaaagatcaaaggatcttcttgagatcctttttttctgcgcgtaatctgctgcttgcaaacaaaaaaaccaccgctaccagcggtggtttgtttgccggatcaagagctaccaactctttttccgaaggtaactggcttcagcagagcgcagataccaaatactgttcttctagtgtagccgtagttaggccaccacttcaagaactctgtagcaccgcctacatacctcgctctgctaatcctgttaccagtggctgctgccagtggcgataagtcgtgtcttaccgggttggactcaagacgatagttaccggataaggcgcagcggtcgggctgaacggggggttcgtgcacacagcccagcttggagcgaacgacctacaccgaactgagatacctacagcgtgagctatgagaaagcgccacgcttcccgaagggagaaaggcggacaggtatccggtaagcggcagggtcggaacaggagagcgcacgagggagcttccagggggaaacgcctggtatctttatagtcctgtcgggtttcgccacctctgacttgagcgtcgatttttgtgatgctcgtcaggggggcggagcctatggaaaaacgccagcaacgcggcctttttacggttcctggccttttgctggccttttgctcacatgttctt

SEQ ID NO: 5 - DNA, 20 bp, Artificial
  Primer
ctacatgcaccagcaactgt

SEQ ID NO: 6 - DNA, 20 bp, Artificial
  Primer
cacctgtgcctgttaaacca

SEQ ID NO: 7 - DNA, 20 bp, Artificial
  Primer
agccagagcatcatcgccta

SEQ ID NO: 8 - DNA, 20 bp, Artificial
  Primer
tggtcacgctgatggtgaag

SEQ ID NO: 9 - DNA, 20 bp, Artificial
  Primer
gcaccgtcaaggctgagaac

SEQ ID NO: 10 - DNA, 19 bp, Artificial
  Primer
tggtgaagacgccagtgga

SEQ ID NO: 11 - protein, 1254 aa, Artificial
  An amino acid sequence of modified SARS-CoV-2 spike protein (4GP)
MFVFLVLLPLVSSQCVNLTTRTQLPPAYTNSFTRGVYYPDKVFRSSVLHSTQDLFLPFFSNVTWFHAIHVSGTNGTKRFDNPVLPFNDGVYFASTEKSNIIRGWIFGTTLDSKTQSLLIVNNATNVVIKVCEFQFCNDPFLGVYYHKNNKSWMESEFRVYSSANNCTFEYVSQPFLMDLEGKQGNFKNLREFVFKNIDGYFKIYSKHTPINLVRDLPQGFSALEPLVDLPIGINITRFQTLLALHRSYLTPGDSSSGWTAGAAAYYVGYLQPRTFLLKYNENGTITDAVDCALDPLSETKCTLKSFTVEKGIYQTSNFRVQPTESIVRFPNITNLCPFGEVFNATRFASVYAWNRKRISNCVADYSVLYNSASFSTFKCYGVSPTKLNDLCFTNVYADSFVIRGDEVRQIAPGQTGKIADYNYKLPDDFTGCVIAWNSNNLDSKVGGNYNYLYRLFRKSNLKPFERDISTEIYQAGSTPCNGVEGFNCYFPLQSYGFQPTNGVGYQPYRVVVLSFELLHAPATVCGPKKSTNLVKNKCVNFNFNGLTGTGVLTESNKKFLPFQQFGRDIADTTDAVRDPQTLEILDITPCSFGGVSVITPGTNTSNQVAVLYQGVNCTEVPVAIHADQLTPTWRVYSTGSNVFQTRAGCLIGAEHVNNSYECDIPIGAGICASYQTQTNSPRRARSVASQSIIAYTMSLGAENSVAYSNNSIAIPTNFTISVTTEILPVSMTKTSVDCTMYICGDSTECSNLLLQYGSFCTQLNRALTGIAVEQDKNTQEVFAQVKQIYKTPPIKDFGGFNFSQILPDPSKPSKRSFIEDLLFNKVTLADAGFIKQYGDCLGDIAARDLICAQKFNGLTVLPPLLTDEMIAQYTSALLAGTITSGWTFGAGAALQIPFAMQMAYRFNGIGVTQNVLYENQKLIANQFNSAIGKIQDSLSSTASALGKLQDVVNQNAQALNTLVKQLSSNFGAISSVLNDILSRLDPPEAEVQIDRLITGRLQSLQTYVTQQLIRAAEIRASANLAATKMSECVLGQSKRVDFCGKGYHLMSFPQSAPHGVVFLHVTYVPAQEKNFTTAPAICHDGKAHFPREGVFVSNGTHWFVTQRNFYEPQIITTDNTFVSGNCDVVIGIVNNTVYDPLQPELDSFKEELDKYFKNHTSPDVDLGDISGINASVVNIQKEIDRLNEVAKNLNESLIDLQELGKYEQYIKWPWYIWLGFIAGLIAIVMVTIMLCCMTSCCSCLKGCCSCGSCC

SEQ ID NO: 12 - DNA, 3765 bp, Artificial
  A nucleotide sequence coding modified SARS-CoV-2 spike protein (4GP)
atgttcgtgttcctggtgctgctgcccctggtgagcagccagtgcgtgaacctgaccaccagaacccagctgccccccgcctacaccaacagcttcaccagaggcgtgtactaccccgacaaggtgttcagaagcagcgtgctgcacagcacccaggacctgttcctgcccttcttcagcaacgtgacctggttccacgccatccacgtgagcggcaccaacggcaccaagagattcgacaaccccgtgctgcccttcaacgacggcgtgtacttcgccagcaccgagaagagcaacatcatcagaggctggatcttcggcaccaccctggacagcaagacccagagcctgctgatcgtgaacaacgccaccaacgtggtgatcaaggtgtgcgagttccagttctgcaacgaccccttcctgggcgtgtactaccacaagaacaacaagagctggatggagagcgagttcagagtgtacagcagcgccaacaactgcaccttcgagtacgtgagccagcccttcctgatggacctggagggcaagcagggcaacttcaagaacctgagagagttcgtgttcaagaacatcgacggctacttcaagatctacagcaagcacacccccatcaacctggtgagagacctgcctcagggctttagcgccctggagccactggtggacctgccaatcggcatcaacatcaccagattccagaccctgctggccctgcacagaagctacctgacaccaggcgattctagctctggatggacagccggcgccgctgcctattacgtgggctacctgcagcctagaaccttcctgctgaagtacaacgagaacggcaccatcaccgatgccgtggactgcgccctggatcccctgagcgagaccaagtgtaccctgaagagcttcaccgtggagaagggcatctaccagaccagcaacttcagagtgcagcccaccgagagcatcgtgagattccccaacatcaccaacctgtgccccttcggcgaggtgttcaacgccaccagattcgccagcgtgtacgcctggaacagaaagagaatcagcaactgcgtggccgactacagcgtgctgtacaacagcgccagcttcagcaccttcaagtgctacggcgtgagccccaccaagctgaacgacctgtgcttcaccaacgtgtacgccgacagcttcgtgatcagaggcgacgaggtgagacagattgcccctggccagaccggcaagatcgccgactacaactacaagctgcccgacgacttcaccggctgcgtgatcgcctggaacagcaacaacctggacagcaaggtgggcggcaactacaactacctgtacagactgttcagaaagagcaacctgaagcccttcgagagagacatcagcaccgagatctaccaggccggctctaccccatgcaatggcgtggagggcttcaattgctacttccccctgcagagctacggcttccagcccaccaacggcgtgggctaccagccctacagagtggtggtgctgagctttgaactgctgcacgcccctgccaccgtgtgcggcccaaagaagagcaccaatctggtgaagaacaagtgcgtgaacttcaacttcaacggcctgaccggcaccggcgtgctgaccgagagcaacaagaagttcctgcccttccagcagttcggcagagacatcgccgacaccaccgatgccgtgagagatccccagaccctggagatcctggacatcaccccctgtagctttggcggcgtgagcgtgattacccccggcaccaataccagcaaccaggtggccgtgctgtaccagggcgtgaactgcaccgaggtgccagtggccatccatgccgaccagctgaccccaacctggagagtgtacagcaccggcagcaacgtgttccagacaagagccggctgtctgattggcgccgagcacgtgaataacagctacgagtgcgatatcccaatcggcgccggcatctgtgccagctatcagacccagaccaatagccccagaagagccagaagcgtggccagccagagcatcatcgcctacaccatgagcctgggcgccgagaacagcgtggcctacagcaacaacagcatcgccatccccaccaacttcaccatcagcgtgaccaccgagatcctgcccgtgagcatgaccaagaccagcgtggactgcaccatgtacatctgcggcgacagcaccgagtgcagcaacctgctgctgcagtacggcagcttctgcacccagctgaacagagccctgaccggcatcgccgtggagcaggacaagaacacccaggaggtgttcgcccaggtgaagcagatctacaagaccccccccatcaaggacttcggcggcttcaacttcagccagatcctgcccgaccccagcaagcccagcaagagaagcttcatcgaggacctgctgttcaacaaggtgaccctggccgacgccggcttcatcaagcagtacggcgactgcctgggcgacatcgccgccagagacctgatctgcgcccagaagtttaatggactgacagtgctgccacccctgctgaccgatgagatgatcgcccagtacaccagcgctctgctggccggcacaatcaccagcggctggacatttggagccggagccgctctgcagatcccatttgccatgcagatggcctacagattcaacggcatcggcgtgacccagaacgtgctgtacgagaaccagaagctgatcgccaaccagttcaacagcgccatcggcaagatccaggacagcctgtctagcacagcctctgccctgggcaagctgcaggatgtggtgaaccagaacgcccaggccctgaacaccctggtgaagcagctgagcagcaacttcggcgccatcagcagcgtgctgaacgacatcctgagcagactggacccccctgaggccgaggtgcagatcgacagactgatcaccggcagactgcagagcctgcagacctacgtgacccagcagctgatcagagccgccgaaatcagagccagcgccaatctggccgccaccaagatgagcgagtgcgtgctgggccagagcaagagagtggacttctgcggcaagggctaccacctgatgagctttccccagagcgcccctcacggcgtggtgtttctgcacgtgacctacgtgcctgcccaggagaagaacttcaccaccgcccctgccatctgccacgatggcaaggcccacttccctagagagggcgtgttcgtgagcaacggcacccactggttcgtgacccagagaaacttctacgagccccagatcatcaccaccgacaacaccttcgtgagcggcaactgcgacgtggtgatcggcatcgtgaacaacaccgtgtacgaccccctgcagcccgagctggacagcttcaaggaggagctggacaagtacttcaagaaccacaccagccccgatgtggacctgggcgatatcagcggcatcaatgccagcgtggtgaacatccagaaggagatcgaccggctcaatgaggtggccaagaacctgaacgagagcctgatcgacctgcaggaactgggcaaatatgagcagtacatcaagtggccctggtacatctggctgggcttcatcgccggcctgatcgccatcgtgatggtgaccatcatgctgtgctgcatgaccagctgctgcagctgcctgaagggctgctgcagctgcgggtcttgttgctaa

SEQ ID NO: 13 - protein, 1254 aa, Artificial
  An amino acid sequence of modified SARS-CoV-2 spike protein (SA)
MFVFLVLLPLVSSQCVNFTTRTQLPPAYTNSFTRGVYYPDKVFRSSVLHSTQDLFLPFFSNVTWFHAIHVSGTNGTKRFANPVLPFNDGVYFASTEKSNIIRGWIFGTTLDSKTQSLLIVNNATNVVIKVCEFQFCNDPFLGVYYHKNNKSWMESEFRVYSSANNCTFEYVSQPFLMDLEGKQGNFKNLREFVFKNIDGYFKIYSKHTPINLVRGLPQGFSALEPLVDLPIGINITRFQTLLALHISYLTPGDSSSGWTAGAAAYYVGYLQPRTFLLKYNENGTITDAVDCALDPLSETKCTLKSFTVEKGIYQTSNFRVQPTESIVRFPNITNLCPFGEVFNATRFASVYAWNRKRISNCVADYSVLYNSASFSTFKCYGVSPTKLNDLCFTNVYADSFVIRGDEVRQIAPGQTGNIADYNYKLPDDFTGCVIAWNSNNLDSKVGGNYNYLYRLFRKSNLKPFERDISTEIYQAGSTPCNGVKGFNCYFPLQSYGFQPTYGVGYQPYRVVVLSFELLHAPATVCGPKKSTNLVKNKCVNFNFNGLTGTGVLTESNKKFLPFQQFGRDIADTTDAVRDPQTLEILDITPCSFGGVSVITPGTNTSNQVAVLYQGVNCTEVPVAIHADQLTPTWRVYSTGSNVFQTRAGCLIGAEHVNNSYECDIPIGAGICASYQTQTNSPRRARSVASQSIIAYTMSLGVENSVAYSNNSIAIPTNFTISVTTEILPVSMTKTSVDCTMYICGDSTECSNLLLQYGSFCTQLNRALTGIAVEQDKNTQEVFAQVKQIYKTPPIKDFGGFNFSQILPDPSKPSKRSFIEDLLFNKVTLADAGFIKQYGDCLGDIAARDLICAQKFNGLTVLPPLLTDEMIAQYTSALLAGTITSGWTFGAGAALQIPFAMQMAYRFNGIGVTQNVLYENQKLIANQFNSAIGKIQDSLSSTASALGKLQDVVNQNAQALNTLVKQLSSNFGAISSVLNDILSRLDPPEAEVQIDRLITGRLQSLQTYVTQQLIRAAEIRASANLAATKMSECVLGQSKRVDFCGKGYHLMSFPQSAPHGVVFLHVTYVPAQEKNFTTAPAICHDGKAHFPREGVFVSNGTHWFVTQRNFYEPQIITTDNTFVSGNCDVVIGIVNNTVYDPLQPELDSFKEELDKYFKNHTSPDVDLGDISGINASVVNIQKEIDRLNEVAKNLNESLIDLQELGKYEQYIKWPWYIWLGFIAGLIAIVMVTIMLCCMTSCCSCLKGCCSCGSCC

SEQ ID NO: 14 - DNA, 3765 bp, Artificial
  A nucleotide sequence coding modified SARS-CoV-2 spike protein (SA)
atgttcgtgttcctggtgctgctgcccctggtgagcagccagtgcgtgaacttcaccaccagaacccagctgccccccgcctacaccaacagcttcaccagaggcgtgtactaccccgacaaggtgttcagaagcagcgtgctgcacagcacccaggacctgttcctgcccttcttcagcaacgtgacctggttccacgccatccacgtgagcggcaccaacggcaccaagagattcgccaaccccgtgctgcccttcaacgacggcgtgtacttcgccagcaccgagaagagcaacatcatcagaggctggatcttcggcaccaccctggacagcaagacccagagcctgctgatcgtgaacaacgccaccaacgtggtgatcaaggtgtgcgagttccagttctgcaacgaccccttcctgggcgtgtactaccacaagaacaacaagagctggatggagagcgagttcagagtgtacagcagcgccaacaactgcaccttcgagtacgtgagccagcccttcctgatggacctggagggcaagcagggcaacttcaagaacctgagagagttcgtgttcaagaacatcgacggctacttcaagatctacagcaagcacacccccatcaacctggtgagaggcctgcctcagggctttagcgccctggagccactggtggacctgccaatcggcatcaacatcaccagattccagaccctgctggccctgcacatcagctacctgacaccaggcgattctagctctggatggacagccggcgccgctgcctattacgtgggctacctgcagcctagaaccttcctgctgaagtacaacgagaacggcaccatcaccgatgccgtggactgcgccctggatcccctgagcgagaccaagtgtaccctgaagagcttcaccgtggagaagggcatctaccagaccagcaacttcagagtgcagcccaccgagagcatcgtgagattccccaacatcaccaacctgtgccccttcggcgaggtgttcaacgccaccagattcgccagcgtgtacgcctggaacagaaagagaatcagcaactgcgtggccgactacagcgtgctgtacaacagcgccagcttcagcaccttcaagtgctacggcgtgagccccaccaagctgaacgacctgtgcttcaccaacgtgtacgccgacagcttcgtgatcagaggcgacgaggtgagacagattgcccctggccagaccggcaacatcgccgactacaactacaagctgcccgacgacttcaccggctgcgtgatcgcctggaacagcaacaacctggacagcaaggtgggcggcaactacaactacctgtacagactgttcagaaagagcaacctgaagcccttcgagagagacatcagcaccgagatctaccaggccggctctaccccatgcaatggcgtgaagggcttcaattgctacttccccctgcagagctacggcttccagcccacctacggcgtgggctaccagccctacagagtggtggtgctgagctttgaactgctgcacgcccctgccaccgtgtgcggcccaaagaagagcaccaatctggtgaagaacaagtgcgtgaacttcaacttcaacggcctgaccggcaccggcgtgctgaccgagagcaacaagaagttcctgcccttccagcagttcggcagagacatcgccgacaccaccgatgccgtgagagatccccagaccctggagatcctggacatcaccccctgtagctttggcggcgtgagcgtgattacccccggcaccaataccagcaaccaggtggccgtgctgtaccagggcgtgaactgcaccgaggtgccagtggccatccatgccgaccagctgaccccaacctggagagtgtacagcaccggcagcaacgtgttccagacaagagccggctgtctgattggcgccgagcacgtgaataacagctacgagtgcgatatcccaatcggcgccggcatctgtgccagctatcagacccagaccaatagccccagaagagccagaagcgtggccagccagagcatcatcgcctacaccatgagcctgggcgtggagaacagcgtggcctacagcaacaacagcatcgccatccccaccaacttcaccatcagcgtgaccaccgagatcctgcccgtgagcatgaccaagaccagcgtggactgcaccatgtacatctgcggcgacagcaccgagtgcagcaacctgctgctgcagtacggcagcttctgcacccagctgaacagagccctgaccggcatcgccgtggagcaggacaagaacacccaggaggtgttcgcccaggtgaagcagatctacaagaccccccccatcaaggacttcggcggcttcaacttcagccagatcctgcccgaccccagcaagcccagcaagagaagcttcatcgaggacctgctgttcaacaaggtgaccctggccgacgccggcttcatcaagcagtacggcgactgcctgggcgacatcgccgccagagacctgatctgcgcccagaagtttaatggactgacagtgctgccacccctgctgaccgatgagatgatcgcccagtacaccagcgctctgctggccggcacaatcaccagcggctggacatttggagccggagccgctctgcagatcccatttgccatgcagatggcctacagattcaacggcatcggcgtgacccagaacgtgctgtacgagaaccagaagctgatcgccaaccagttcaacagcgccatcggcaagatccaggacagcctgtctagcacagcctctgccctgggcaagctgcaggatgtggtgaaccagaacgcccaggccctgaacaccctggtgaagcagctgagcagcaacttcggcgccatcagcagcgtgctgaacgacatcctgagcagactggacccccctgaggccgaggtgcagatcgacagactgatcaccggcagactgcagagcctgcagacctacgtgacccagcagctgatcagagccgccgaaatcagagccagcgccaatctggccgccaccaagatgagcgagtgcgtgctgggccagagcaagagagtggacttctgcggcaagggctaccacctgatgagctttccccagagcgcccctcacggcgtggtgtttctgcacgtgacctacgtgcctgcccaggagaagaacttcaccaccgcccctgccatctgccacgatggcaaggcccacttccctagagagggcgtgttcgtgagcaacggcacccactggttcgtgacccagagaaacttctacgagccccagatcatcaccaccgacaacaccttcgtgagcggcaactgcgacgtggtgatcggcatcgtgaacaacaccgtgtacgaccccctgcagcccgagctggacagcttcaaggaggagctggacaagtacttcaagaaccacaccagccccgatgtggacctgggcgatatcagcggcatcaatgccagcgtggtgaacatccagaaggagatcgaccggctcaatgaggtggccaagaacctgaacgagagcctgatcgacctgcaggaactgggcaaatatgagcagtacatcaagtggccctggtacatctggctgggcttcatcgccggcctgatcgccatcgtgatggtgaccatcatgctgtgctgcatgaccagctgctgcagctgcctgaagggctgctgcagctgcgggtcttgttgctaa

SEQ ID NO: 15 - protein, 1254 aa, Artificial
  An amino acid sequence of modified SARS-CoV-2 spike protein (BR)
MFVFLVLLPLVSSQCVNFTNRTQLPSAYTNSFTRGVYYPDKVFRSSVLHSTQDLFLPFFSNVTWFHAIHVSGTNGTKRFDNPVLPFNDGVYFASTEKSNIIRGWIFGTTLDSKTQSLLIVNNATNVVIKVCEFQFCNYPFLGVYYHKNNKSWMESEFRVYSSANNCTFEYVSQPFLMDLEGKQGNFKNLSEFVFKNIDGYFKIYSKHTPINLVRDLPQGFSALEPLVDLPIGINITRFQTLLALHRSYLTPGDSSSGWTAGAAAYYVGYLQPRTFLLKYNENGTITDAVDCALDPLSETKCTLKSFTVEKGIYQTSNFRVQPTESIVRFPNITNLCPFGEVFNATRFASVYAWNRKRISNCVADYSVLYNSASFSTFKCYGVSPTKLNDLCFTNVYADSFVIRGDEVRQIAPGQTGTIADYNYKLPDDFTGCVIAWNSNNLDSKVGGNYNYLYRLFRKSNLKPFERDISTEIYQAGSTPCNGVKGFNCYFPLQSYGFQPTYGVGYQPYRVVVLSFELLHAPATVCGPKKSTNLVKNKCVNFNFNGLTGTGVLTESNKKFLPFQQFGRDIADTTDAVRDPQTLEILDITPCSFGGVSVITPGTNTSNQVAVLYQGVNCTEVPVAIHADQLTPTWRVYSTGSNVFQTRAGCLIGAEYVNNSYECDIPIGAGICASYQTQTNSPRRARSVASQSIIAYTMSLGAENSVAYSNNSIAIPTNFTISVTTEILPVSMTKTSVDCTMYICGDSTECSNLLLQYGSFCTQLNRALTGIAVEQDKNTQEVFAQVKQIYKTPPIKDFGGFNFSQILPDPSKPSKRSFIEDLLFNKVTLADAGFIKQYGDCLGDIAARDLICAQKFNGLTVLPPLLTDEMIAQYTSALLAGTITSGWTFGAGAALQIPFAMQMAYRFNGIGVTQNVLYENQKLIANQFNSAIGKIQDSLSSTASALGKLQDVVNQNAQALNTLVKQLSSNFGAISSVLNDILSRLDPPEAEVQIDRLITGRLQSLQTYVTQQLIRAAEIRASANLAAYKMSECVLGQSKRVDFCGKGYHLMSFPQSAPHGVVFLHVTYVPAQEKNFTTAPAICHDGKAHFPREGVFVSNGTHWFVTQRNFYEPQIITTDNTFVSGNCDVVIGIVNNTVYDPLQPELDSFKEELDKYFKNHTSPDVDLGDISGINASFVNIQKEIDRLNEVAKNLNESLIDLQELGKYEQYIKWPWYIWLGFIAGLIAIVMVTIMLCCMTSCCSCLKGCCSCGSCC

SEQ ID NO: 16 - DNA, 3765 bp, Artificial
  A nucleotide sequence coding modified SARS-CoV-2 spike protein (BR)
atgttcgtgttcctggtgctgctgcccctggtgagcagccagtgcgtgaacttcaccaacagaacccagctgcccagcgcctacaccaacagcttcaccagaggcgtgtactaccccgacaaggtgttcagaagcagcgtgctgcacagcacccaggacctgttcctgcccttcttcagcaacgtgacctggttccacgccatccacgtgagcggcaccaacggcaccaagagattcgacaaccccgtgctgcccttcaacgacggcgtgtacttcgccagcaccgagaagagcaacatcatcagaggctggatcttcggcaccaccctggacagcaagacccagagcctgctgatcgtgaacaacgccaccaacgtggtgatcaaggtgtgcgagttccagttctgcaactaccccttcctgggcgtgtactaccacaagaacaacaagagctggatggagagcgagttcagagtgtacagcagcgccaacaactgcaccttcgagtacgtgagccagcccttcctgatggacctggagggcaagcagggcaacttcaagaacctgagcgagttcgtgttcaagaacatcgacggctacttcaagatctacagcaagcacacccccatcaacctggtgagagacctgcctcagggctttagcgccctggagccactggtggacctgccaatcggcatcaacatcaccagattccagaccctgctggccctgcacagaagctacctgacaccaggcgattctagctctggatggacagccggcgccgctgcctattacgtgggctacctgcagcctagaaccttcctgctgaagtacaacgagaacggcaccatcaccgatgccgtggactgcgccctggatcccctgagcgagaccaagtgtaccctgaagagcttcaccgtggagaagggcatctaccagaccagcaacttcagagtgcagcccaccgagagcatcgtgagattccccaacatcaccaacctgtgccccttcggcgaggtgttcaacgccaccagattcgccagcgtgtacgcctggaacagaaagagaatcagcaactgcgtggccgactacagcgtgctgtacaacagcgccagcttcagcaccttcaagtgctacggcgtgagccccaccaagctgaacgacctgtgcttcaccaacgtgtacgccgacagcttcgtgatcagaggcgacgaggtgagacagattgcccctggccagaccggcaccatcgccgactacaactacaagctgcccgacgacttcaccggctgcgtgatcgcctggaacagcaacaacctggacagcaaggtgggcggcaactacaactacctgtacagactgttcagaaagagcaacctgaagcccttcgagagagacatcagcaccgagatctaccaggccggctctaccccatgcaatggcgtgaagggcttcaattgctacttccccctgcagagctacggcttccagcccacctacggcgtgggctaccagccctacagagtggtggtgctgagctttgaactgctgcacgcccctgccaccgtgtgcggcccaaagaagagcaccaatctggtgaagaacaagtgcgtgaacttcaacttcaacggcctgaccggcaccggcgtgctgaccgagagcaacaagaagttcctgcccttccagcagttcggcagagacatcgccgacaccaccgatgccgtgagagatccccagaccctggagatcctggacatcaccccctgtagctttggcggcgtgagcgtgattacccccggcaccaataccagcaaccaggtggccgtgctgtaccagggcgtgaactgcaccgaggtgccagtggccatccatgccgaccagctgaccccaacctggagagtgtacagcaccggcagcaacgtgttccagacaagagccggctgtctgattggcgccgagtacgtgaataacagctacgagtgcgatatcccaatcggcgccggcatctgtgccagctatcagacccagaccaatagccccagaagagccagaagcgtggccagccagagcatcatcgcctacaccatgagcctgggcgccgagaacagcgtggcctacagcaacaacagcatcgccatccccaccaacttcaccatcagcgtgaccaccgagatcctgcccgtgagcatgaccaagaccagcgtggactgcaccatgtacatctgcggcgacagcaccgagtgcagcaacctgctgctgcagtacggcagcttctgcacccagctgaacagagccctgaccggcatcgccgtggagcaggacaagaacacccaggaggtgttcgcccaggtgaagcagatctacaagaccccccccatcaaggacttcggcggcttcaacttcagccagatcctgcccgaccccagcaagcccagcaagagaagcttcatcgaggacctgctgttcaacaaggtgaccctggccgacgccggcttcatcaagcagtacggcgactgcctgggcgacatcgccgccagagacctgatctgcgcccagaagtttaatggactgacagtgctgccacccctgctgaccgatgagatgatcgcccagtacaccagcgctctgctggccggcacaatcaccagcggctggacatttggagccggagccgctctgcagatcccatttgccatgcagatggcctacagattcaacggcatcggcgtgacccagaacgtgctgtacgagaaccagaagctgatcgccaaccagttcaacagcgccatcggcaagatccaggacagcctgtctagcacagcctctgccctgggcaagctgcaggatgtggtgaaccagaacgcccaggccctgaacaccctggtgaagcagctgagcagcaacttcggcgccatcagcagcgtgctgaacgacatcctgagcagactggacccccctgaggccgaggtgcagatcgacagactgatcaccggcagactgcagagcctgcagacctacgtgacccagcagctgatcagagccgccgaaatcagagccagcgccaatctggccgccatcaagatgagcgagtgcgtgctgggccagagcaagagagtggacttctgcggcaagggctaccacctgatgagctttccccagagcgcccctcacggcgtggtgtttctgcacgtgacctacgtgcctgcccaggagaagaacttcaccaccgcccctgccatctgccacgatggcaaggcccacttccctagagagggcgtgttcgtgagcaacggcacccactggttcgtgacccagagaaacttctacgagccccagatcatcaccaccgacaacaccttcgtgagcggcaactgcgacgtggtgatcggcatcgtgaacaacaccgtgtacgaccccctgcagcccgagctggacagcttcaaggaggagctggacaagtacttcaagaaccacaccagccccgatgtggacctgggcgatatcagcggcatcaatgccagcttcgtgaacatccagaaggagatcgaccggctcaatgaggtggccaagaacctgaacgagagcctgatcgacctgcaggaactgggcaaatatgagcagtacatcaagtggccctggtacatctggctgggcttcatcgccggcctgatcgccatcgtgatggtgaccatcatgctgtgctgcatgaccagctgctgcagctgcctgaagggctgctgcagctgcgggtcttgttgctaa

SEQ ID NO: 17 - protein, 1252 aa, Artificial
  An amino acid sequence of modified SARS-CoV-2 spike protein (IN)
MFVFLVLLPLVSSQCVNLRTRTQLPPAYTNSFTRGVYYPDKVFRSSVLHSTQDLFLPFFSNVTWFHAIHVSGTNGTKRFDNPVLPFNDGVYFASTEKSNIIRGWIFGTTLDSKTQSLLIVNNATNVVIKVCEFQFCNDPFLDVYYHKNNKSWMESGVYSSANNCTFEYVSQPFLMDLEGKQGNFKNLREFVFKNIDGYFKIYSKHTPINLVRDLPQGFSALEPLVDLPIGINITRFQTLLALHRSYLTPGDSSSGWTAGAAAYYVGYLQPRTFLLKYNENGTITDAVDCALDPLSETKCTLKSFTVEKGIYQTSNFRVQPTESIVRFPNITNLCPFGEVFNATRFASVYAWNRKRISNCVADYSVLYNSASFSTFKCYGVSPTKLNDLCFTNVYADSFVIRGDEVRQIAPGQTGKIADYNYKLPDDFTGCVIAWNSNNLDSKVGGNYNYRYRLFRKSNLKPFERDISTEIYQAGSKPCNGVEGFNCYFPLQSYGFQPTNGVGYQPYRVVVLSFELLHAPATVCGPKKSTNLVKNKCVNFNFNGLTGTGVLTESNKKFLPFQQFGRDIADTTDAVRDPQTLEILDITPCSFGGVSVITPGTNTSNQVAVLYQGVNCTEVPVAIHADQLTPTWRVYSTGSNVFQTRAGCLIGAEHVNNSYECDIPIGAGICASYQTQTNSRRRARSVASQSIIAYTMSLGAENSVAYSNNSIAIPTNFTISVTTEILPVSMTKTSVDCTMYICGDSTECSNLLLQYGSFCTQLNRALTGIAVEQDKNTQEVFAQVKQIYKTPPIKDFGGFNFSQILPDPSKPSKRSFIEDLLFNKVTLADAGFIKQYGDCLGDIAARDLICAQKFNGLTVLPPLLTDEMIAQYTSALLAGTITSGWTFGAGAALQIPFAMQMAYRFNGIGVTQNVLYENQKLIANQFNSAIGKIQDSLSSTASALGKLQNVVNQNAQALNTLVKQLSSNFGAISSVLNDILSRLDPPEAEVQIDRLITGRLQSLQTYVTQQLIRAAEIRASANLAATKMSECVLGQSKRVDFCGKGYHLMSFPQSAPHGVVFLHVTYVPAQEKNFTTAPAICHDGKAHFPREGVFVSNGTHWFVTQRNFYEPQIITTDNTFVSGNCDVVIGIVNNTVYDPLQPELDSFKEELDKYFKNHTSPDVDLGDISGINASVVNIQKEIDRLNEVAKNLNESLIDLQELGKYEQYIKWPWYIWLGFIAGLIAIVMVTIMLCCMTSCCSCLKGCCSCGSCC

SEQ ID NO: 18 - DNA, 3759 bp, Artificial
  A nucleotide sequence coding modified SARS-CoV-2 spike protein (IN)
atgttcgtgttcctggtgctgctgcccctggtgagcagccagtgcgtgaacctgagaaccagaacccagctgccccccgcctacaccaacagcttcaccagaggcgtgtactaccccgacaaggtgttcagaagcagcgtgctgcacagcacccaggacctgttcctgcccttcttcagcaacgtgacctggttccacgccatccacgtgagcggcaccaacggcaccaagagattcgacaaccccgtgctgcccttcaacgacggcgtgtacttcgccagcaccgagaagagcaacatcatcagaggctggatcttcggcaccaccctggacagcaagacccagagcctgctgatcgtgaacaacgccaccaacgtggtgatcaaggtgtgcgagttccagttctgcaacgaccccttcctggacgtgtactaccacaagaacaacaagagctggatggagagcggcgtgtacagcagcgccaacaactgcaccttcgagtacgtgagccagcccttcctgatggacctggagggcaagcagggcaacttcaagaacctgagagagttcgtgttcaagaacatcgacggctacttcaagatctacagcaagcacacccccatcaacctggtgagagacctgcctcagggctttagcgccctggagccactggtggacctgccaatcggcatcaacatcaccagattccagaccctgctggccctgcacagaagctacctgacaccaggcgattctagctctggatggacagccggcgccgctgcctattacgtgggctacctgcagcctagaaccttcctgctgaagtacaacgagaacggcaccatcaccgatgccgtggactgcgccctggatcccctgagcgagaccaagtgtaccctgaagagcttcaccgtggagaagggcatctaccagaccagcaacttcagagtgcagcccaccgagagcatcgtgagattccccaacatcaccaacctgtgccccttcggcgaggtgttcaacgccaccagattcgccagcgtgtacgcctggaacagaaagagaatcagcaactgcgtggccgactacagcgtgctgtacaacagcgccagcttcagcaccttcaagtgctacggcgtgagccccaccaagctgaacgacctgtgcttcaccaacgtgtacgccgacagcttcgtgatcagaggcgacgaggtgagacagattgcccctggccagaccggcaagatcgccgactacaactacaagctgcccgacgacttcaccggctgcgtgatcgcctggaacagcaacaacctggacagcaaggtgggcggcaactacaactacagatacagactgttcagaaagagcaacctgaagcccttcgagagagacatcagcaccgagatctaccaggccggctctaagccatgcaatggcgtggagggcttcaattgctacttccccctgcagagctacggcttccagcccaccaacggcgtgggctaccagccctacagagtggtggtgctgagctttgaactgctgcacgcccctgccaccgtgtgcggcccaaagaagagcaccaatctggtgaagaacaagtgcgtgaacttcaacttcaacggcctgaccggcaccggcgtgctgaccgagagcaacaagaagttcctgcccttccagcagttcggcagagacatcgccgacaccaccgatgccgtgagagatccccagaccctggagatcctggacatcaccccctgtagctttggcggcgtgagcgtgattacccccggcaccaataccagcaaccaggtggccgtgctgtaccagggcgtgaactgcaccgaggtgccagtggccatccatgccgaccagctgaccccaacctggagagtgtacagcaccggcagcaacgtgttccagacaagagccggctgtctgattggcgccgagcacgtgaataacagctacgagtgcgatatcccaatcggcgccggcatctgtgccagctatcagacccagaccaatagcagaagaagagccagaagcgtggccagccagagcatcatcgcctacaccatgagcctgggcgccgagaacagcgtggcctacagcaacaacagcatcgccatccccaccaacttcaccatcagcgtgaccaccgagatcctgcccgtgagcatgaccaagaccagcgtggactgcaccatgtacatctgcggcgacagcaccgagtgcagcaacctgctgctgcagtacggcagcttctgcacccagctgaacagagccctgaccggcatcgccgtggagcaggacaagaacacccaggaggtgttcgcccaggtgaagcagatctacaagaccccccccatcaaggacttcggcggcttcaacttcagccagatcctgcccgaccccagcaagcccagcaagagaagcttcatcgaggacctgctgttcaacaaggtgaccctggccgacgccggcttcatcaagcagtacggcgactgcctgggcgacatcgccgccagagacctgatctgcgcccagaagtttaatggactgacagtgctgccacccctgctgaccgatgagatgatcgcccagtacaccagcgctctgctggccggcacaatcaccagcggctggacatttggagccggagccgctctgcagatcccatttgccatgcagatggcctacagattcaacggcatcggcgtgacccagaacgtgctgtacgagaaccagaagctgatcgccaaccagttcaacagcgccatcggcaagatccaggacagcctgtctagcacagcctctgccctgggcaagctgcagaacgtggtgaaccagaacgcccaggccctgaacaccctggtgaagcagctgagcagcaacttcggcgccatcagcagcgtgctgaacgacatcctgagcagactggacccccctgaggccgaggtgcagatcgacagactgatcaccggcagactgcagagcctgcagacctacgtgacccagcagctgatcagagccgccgaaatcagagccagcgccaatctggccgccaccaagatgagcgagtgcgtgctgggccagagcaagagagtggacttctgcggcaagggctaccacctgatgagctttccccagagcgcccctcacggcgtggtgtttctgcacgtgacctacgtgcctgcccaggagaagaacttcaccaccgcccctgccatctgccacgatggcaaggcccacttccctagagagggcgtgttcgtgagcaacggcacccactggttcgtgacccagagaaacttctacgagccccagatcatcaccaccgacaacaccttcgtgagcggcaactgcgacgtggtgatcggcatcgtgaacaacaccgtgtacgaccccctgcagcccgagctggacagcttcaaggaggagctggacaagtacttcaagaaccacaccagccccgatgtggacctgggcgatatcagcggcatcaatgccagcgtggtgaacatccagaaggagatcgaccggctcaatgaggtggccaagaacctgaacgagagcctgatcgacctgcaggaactgggcaaatatgagcagtacatcaagtggccctggtacatctggctgggcttcatcgccggcctgatcgccatcgtgatggtgaccatcatgctgtgctgcatgaccagctgctgcagctgcctgaagggctgctgcagctgcgggtcttgttgctaa